European Patent Application EP 4 140 297 A1, published March 1, 2023. Title: NON-HUMAN ANIMALS HAVING AN ENGINEERED IMMUNOGLOBULIN LAMBDA LIGHT CHAIN AND USES THEREOF. Applicant: REGENERON PHARMACEUTICALS, INC. Application EP. The sequence listing filed with the application follows.

SEQUENCE LISTING (77 sequences)

SEQ ID NO: 1 - DNA, 317 bp, Mus sp.
  source 1..317: mol_type = genomic DNA
gccagcccaagtcttcgccatcagtcaccctgtttccaccttcctctgaagagctcgagactaacaaggccacactggtgtgtacgatcactgatttctacccaggtgtggtgacagtggactggaaggtagatggtacccctgtcactcagggtatggagacaacccagccttccaaacagagcaacaacaagtacatggctagcagctacctgaccctgacagcaagagcatgggaaaggcatagcagttacagctgccaggtcactcatgaaggtcacactgtggagaagagtttgtcccgtgctgactgttcc

SEQ ID NO: 2 - protein, 106 aa, Mus sp.
GQPKSSPSVTLFPPSSEELETNKATLVCTITDFYPGVVTVDWKVDGTPVTQGMETTQPSKQSNNKYMASSYLTLTARAWERHSSYSCQVTHEGHTVEKSLSRADCS

SEQ ID NO: 3 - DNA, 314 bp, Mus sp.
  source 1..314: mol_type = genomic DNA
gtcagcccaagtccactcccactctcaccgtgtttccaccttcctctgaggagctcaaggaaaacaaagccacactggtgtgtctgatttccaacttttccccgagtggtgtgacagtggcctggaaggcaaatggtacacctatcacccagggtgtggacacttcaaatcccaccaaagagggcaacaagttcatggccagcagcttcctacatttgacatcggaccagtggagatctcacaacagttttacctgtcaagttacacatgaaggggacactgtggagaagagtctgtctcctgcagaatgtctc

SEQ ID NO: 4 - protein, 105 aa, Mus sp.
GQPKSTPTLTVFPPSSEELKENKATLVCLISNFSPSGVTVAWKANGTPITQGVDTSNPTKEGNKFMASSFLHLTSDQWRSHNSFTCQVTHEGDTVEKSLSPAECL

SEQ ID NO: 5 - DNA, 314 bp, Mus sp.
  source 1..314: mol_type = genomic DNA
gtcagcccaagtccactcccacactcaccatgtttccaccttcccctgaggagctccaggaaaacaaagccacactcgtgtgtctgatttccaatttttccccaagtggtgtgacagtggcctggaaggcaaatggtacacctatcacccagggtgtggacacttcaaatcccaccaaagaggacaacaagtacatggccagcagcttcttacatttgacatcggaccagtggagatctcacaacagttttacctgccaagttacacatgaaggggacactgtggagaagagtctgtctcctgcagaatgtctc

SEQ ID NO: 6 - protein, 105 aa, Mus sp.
GQPKSTPTLTMFPPSPEELQENKATLVCLISNFSPSGVTVAWKANGTPITQGVDTSNPTKEDNKYMASSFLHLTSDQWRSHNSFTCQVTHEGDTVEKSLSPAECL

SEQ ID NO: 7 - DNA, 314 bp, Rattus sp.
  source 1..314: mol_type = genomic DNA
gtcagcccaagtccactcccacactcacagtatttccaccttcaactgaggagctccagggaaacaaagccacactggtgtgtctgatttctgatttctacccgagtgatgtggaagtggcctggaaggcaaatggtgcacctatctcccagggtgtggacactgcaaatcccaccaaacagggcaacaaatacatcgccagcagcttcttacgtttgacagcagaacagtggagatctcgcaacagttttacctgccaagttacacatgaagggaacactgtggagaagagtctgtctcctgcagaatgtgtc

SEQ ID NO: 8 - protein, 105 aa, Rattus sp.
GQPKSTPTLTVFPPSTEELQGNKATLVCLISDFYPSDVEVAWKANGAPISQGVDTANPTKQGNKYIASSFLRLTAEQWRSRNSFTCQVTHEGNTVEKSLSPAECV

SEQ ID NO: 9 - DNA, 314 bp, Rattus sp.
  source 1..314: mol_type = genomic DNA
accaacccaaggctacgccctcagtcaccctgttcccaccttcctctgaagagctcaagactgacaaggctacactggtgtgtatggtgacagatttctaccctggtgttatgacagtggtctggaaggcagatggtacccctatcactcagggtgtggagactacccagcctttcaaacagaacaacaagtacatggctaccagctacctgcttttgacagcaaaagcatgggagactcatagcaattacagctgccaggtcactcacgaagagaacactgtggagaagagtttgtcccgtgctgagtgttcc

SEQ ID NO: 10 - protein, 105 aa, Rattus sp.
DQPKATPSVTLFPPSSEELKTDKATLVCMVTDFYPGVMTVVWKADGTPITQGVETTQPFKQNNKYMATSYLLLTAKAWETHSNYSCQVTHEENTVEKSLSRAECS

SEQ ID NO: 11 - DNA, 314 bp, Rattus sp.
  source 1..314: mol_type = genomic DNA
gtcagcccaagtccactcccacactcacagtatttccaccttcaactgaggagctccagggaaacaaagccacactggtgtgtctgatttctgatttctacccgagtgatgtggaagtggcctggaaggcaaatggtgcacctatctcccagggtgtggacactgcaaatcccaccaaacagggcaacaaatacatcgccagcagcttcttacgtttgacagcagaacagtggagatctcgcaacagttttacctgccaagttacacatgaagggaacactgtggaaaagagtctgtctcctgcagagtgtgtc

SEQ ID NO: 12 - protein, 105 aa, Rattus sp.; identical to SEQ ID NO: 8

SEQ ID NO: 13 - DNA, 314 bp, Rattus sp.; identical to SEQ ID NO: 9
  source 1..314: mol_type = genomic DNA

SEQ ID NO: 14 - protein, 105 aa, Rattus sp.; identical to SEQ ID NO: 10

SEQ ID NO: 15 - DNA, 315 bp, Homo sapiens
  source 1..315: mol_type = genomic DNA
cccaaggccaaccccacggtcactctgttcccgccctcctctgaggagctccaagccaacaaggccacactagtgtgtctgatcagtgacttctacccgggagctgtgacagtggcttggaaggcagatggcagccccgtcaaggcgggagtggagacgaccaaaccctccaaacagagcaacaacaagtacgcggccagcagctacctgagcctgacgcccgagcagtggaagtcccacagaagctacagctgccaggtcacgcatgaagggagcaccgtggagaagacagtggcccctacagaatgttcatag

SEQ ID NO: 16 - protein, 104 aa, Homo sapiens
PKANPTVTLFPPSSEELQANKATLVCLISDFYPGAVTVAWKADGSPVKAGVETTKPSKQSNNKYAASSYLSLTPEQWKSHRSYSCQVTHEGSTVEKTVAPTECS

SEQ ID NO: 17 - DNA, 317 bp, Homo sapiens
  source 1..317: mol_type = genomic DNA
gtcagcccaaggctgccccctcggtcactctgttcccgccctcctctgaggagcttcaagccaacaaggccacactggtgtgtctcataagtgacttctacccgggagccgtgacagtggcttggaaagcagatagcagccccgtcaaggcgggagtggagaccaccacaccctccaaacaaagcaacaacaagtacgcggccagcagctatctgagcctgacgcctgagcagtggaagtcccacagaagctacagctgccaggtcacgcatgaagggagcaccgtggagaagacagtggcccctacagaatgttca

SEQ ID NO: 18 - protein, 105 aa, Homo sapiens
QPKAAPSVTLFPPSSEELQANKATLVCLISDFYPGAVTVAWKADSSPVKAGVETTTPSKQSNNKYAASSYLSLTPEQWKSHRSYSCQVTHEGSTVEKTVAPTECS

SEQ ID NO: 19 - DNA, 315 bp, Homo sapiens
  source 1..315: mol_type = genomic DNA
cccaaggctgccccctcggtcactctgttcccaccctcctctgaggagcttcaagccaacaaggccacactggtgtgtctcataagtgacttctacccgggagccgtgacagttgcctggaaggcagatagcagccccgtcaaggcgggggtggagaccaccacaccctccaaacaaagcaacaacaagtacgcggccagcagctacctgagcctgacgcctgagcagtggaagtcccacaaaagctacagctgccaggtcacgcatgaagggagcaccgtggagaagacagttgcccctacggaatgttcatag

SEQ ID NO: 20 - protein, 104 aa, Homo sapiens
PKAAPSVTLFPPSSEELQANKATLVCLISDFYPGAVTVAWKADSSPVKAGVETTTPSKQSNNKYAASSYLSLTPEQWKSHKSYSCQVTHEGSTVEKTVAPTECS

SEQ ID NO: 21 - DNA, 321 bp, Homo sapiens
  source 1..321: mol_type = genomic DNA
ggtcagcccaaggctgccccatcggtcactctgttcccgccctcctctgaggagcttcaagccaacaaggccacactggtgtgcctgatcagtgacttctacccgggagctgtgaaagtggcctggaaggcagatggcagccccgtcaacacgggagtggagaccaccacaccctccaaacagagcaacaacaagtacgcggccagcagctacctgagcctgacgcctgagcagtggaagtcccacagaagctacagctgccaggtcacgcatgaagggagcaccgtggagaagacagtggcccctgcagaatgttcatag

SEQ ID NO: 22 - protein, 105 aa, Homo sapiens
QPKAAPSVTLFPPSSEELQANKATLVCLISDFYPGAVKVAWKADGSPVNTGVETTTPSKQSNNKYAASSYLSLTPEQWKSHRSYSCQVTHEGSTVEKTVAPAECS

SEQ ID NO: 23 - DNA, 317 bp, Homo sapiens
  source 1..317: mol_type = genomic DNA
gtcagcccaaggctgccccctcggtcactctgttcccaccctcctctgaggagcttcaagccaacaaggccacactggtgtgtctcgtaagtgacttctacccgggagccgtgacagtggcctggaaggcagatggcagccccgtcaaggtgggagtggagaccaccaaaccctccaaacaaagcaacaacaagtatgcggccagcagctacctgagcctgacgcccgagcagtggaagtcccacagaagctacagctgccgggtcacgcatgaagggagcaccgtggagaagacagtggcccctgcagaatgctct

SEQ ID NO: 24 - protein, 105 aa, Homo sapiens
QPKAAPSVTLFPPSSEELQANKATLVCLVSDFYPGAVTVAWKADGSPVKVGVETTKPSKQSNNKYAASSYLSLTPEQWKSHRSYSCRVTHEGSTVEKTVAPAECS

SEQ ID NO: 25 - DNA, 23 bp, synthetic construct
  misc_feature 1..23: note = Chemically synthesized nucleotide
  source 1..23: mol_type = other DNA
gtggaagattgatggcagtgaac

SEQ ID NO: 26 - DNA, 20 bp, synthetic construct
  misc_feature 1..20: note = Chemically synthesized nucleotide
  source 1..20: mol_type = other DNA
gtgctgctcatgctgtaggt

SEQ ID NO: 27 - DNA, 27 bp, synthetic construct
  misc_feature 1..27: note = Chemically synthesized nucleotide
  source 1..27: mol_type = other DNA
aaatggcgtcctgaacagttggactga

SEQ ID NO: 28 - DNA, 23 bp, synthetic construct
  misc_feature 1..23: note = Chemically synthesized nucleotide
  source 1..23: mol_type = other DNA
ccatccagtgagcagttaacatc

SEQ ID NO: 29 - DNA, 21 bp, synthetic construct
  misc_feature 1..21: note = Chemically synthesized nucleotide
  source 1..21: mol_type = other DNA
tgtcgttcactgccatcaatc

SEQ ID NO: 30 - DNA, 22 bp, synthetic construct
  misc_feature 1..22: note = Chemically synthesized nucleotide
  source 1..22: mol_type = other DNA
aggtgcctcagtcgtgtgcttc

SEQ ID NO: 31 - DNA, 22 bp, synthetic construct
  misc_feature 1..22: note = Chemically synthesized nucleotide
  source 1..22: mol_type = other DNA
ggagcccttccttgttacttca

SEQ ID NO: 32 - DNA, 23 bp, synthetic construct
  misc_feature 1..23: note = Chemically synthesized nucleotide
  source 1..23: mol_type = other DNA
aggtggaaacagggtgactgatg

SEQ ID NO: 33 - DNA, 24 bp, synthetic construct
  misc_feature 1..24: note = Chemically synthesized nucleotide
  source 1..24: mol_type = other DNA
tcctctgtgcttccttcctcaggc

SEQ ID NO: 34 - DNA, 25 bp, synthetic construct
  misc_feature 1..25: note = Chemically synthesized nucleotide
  source 1..25: mol_type = other DNA
tccttgttacttcataccatcctct

SEQ ID NO: 35 - DNA, 22 bp, synthetic construct
  misc_feature 1..22: note = Chemically synthesized nucleotide
  source 1..22: mol_type = other DNA
agggtgactgatggcgaagact

SEQ ID NO: 36 - DNA, 20 bp, synthetic construct
  misc_feature 1..20: note = Chemically synthesized nucleotide
  source 1..20: mol_type = other DNA
ttccttcctcaggccagccc

SEQ ID NO: 37 - DNA, 20 bp, synthetic construct
  misc_feature 1..20: note = Chemically synthesized nucleotide
  source 1..20: mol_type = other DNA
gaggcttgctgagctttcag

SEQ ID NO: 38 - DNA, 18 bp, synthetic construct
  misc_feature 1..18: note = Chemically synthesized nucleotide
  source 1..18: mol_type = other DNA
aggacggtcagcttggtc

SEQ ID NO: 39 - DNA, 25 bp, synthetic construct
  misc_feature 1..25: note = Chemically synthesized nucleotide
  source 1..25: mol_type = other DNA
tatgagcctgtgtcacagtgttggg

SEQ ID NO: 40 - DNA, 20 bp, synthetic construct
  misc_feature 1..20: note = Chemically synthesized nucleotide
  source 1..20: mol_type = other DNA
gctgacccaggactctgttc

SEQ ID NO: 41 - DNA, 23 bp, synthetic construct
  misc_feature 1..23: note = Chemically synthesized nucleotide
  source 1..23: mol_type = other DNA
tcccagttccgaagacataacac

SEQ ID NO: 42 - DNA, 25 bp, synthetic construct
  misc_feature 1..25: note = Chemically synthesized nucleotide
  source 1..25: mol_type = other DNA
ccctttggtgagaagggttttggtc

SEQ ID NO: 43 - DNA, 18 bp, synthetic construct
  misc_feature 1..18: note = Chemically synthesized nucleotide
  source 1..18: mol_type = other DNA
tacgcggccagcagctat

SEQ ID NO: 44 - DNA, 19 bp, synthetic construct
  misc_feature 1..19: note = Chemically synthesized nucleotide
  source 1..19: mol_type = other DNA
tggcagctgtagcttctgt

SEQ ID NO: 45 - DNA, 21 bp, synthetic construct
  misc_feature 1..21: note = Chemically synthesized nucleotide
  source 1..21: mol_type = other DNA
ctgagcctgacgcctgagcag

SEQ ID NO: 46 - DNA, 21 bp, synthetic construct
  misc_feature 1..21: note = Chemically synthesized nucleotide
  source 1..21: mol_type = other DNA
tcaacctttcccagcctgtct

SEQ ID NO: 47 - DNA, 24 bp, synthetic construct
  misc_feature 1..24: note = Chemically synthesized nucleotide
  source 1..24: mol_type = other DNA
ccccagagagagaaaacagatttt

SEQ ID NO: 48 - skipped

SEQ ID NO: 49 - DNA, 16 bp, synthetic construct
  misc_feature 1..16: note = Chemically synthesized nucleotide
  source 1..16: mol_type = other DNA
accctctgctgtccct

SEQ ID NO: 50 - DNA, 19 bp, synthetic construct
  misc_feature 1..19: note = Chemically synthesized nucleotide
  source 1..19: mol_type = other DNA
ggtggagaggctattcggc

SEQ ID NO: 51 - DNA, 17 bp, synthetic construct
  misc_feature 1..17: note = Chemically synthesized nucleotide
  source 1..17: mol_type = other DNA
gaacacggcggcatcag

SEQ ID NO: 52 - DNA, 23 bp, synthetic construct
  misc_feature 1..23: note = Chemically synthesized nucleotide
  source 1..23: mol_type = other DNA
tgggcacaacagacaatcggctg

SEQ ID NO: 53 - DNA, 17 bp, synthetic construct
  misc_feature 1..17: note = Chemically synthesized nucleotide
  source 1..17: mol_type = other DNA
tgcggccgatcttagcc

SEQ ID NO: 54 - DNA, 18 bp, synthetic construct
  misc_feature 1..18: note = Chemically synthesized nucleotide
  source 1..18: mol_type = other DNA
ttgaccgattccttgcgg

SEQ ID NO: 55 - DNA, 21 bp, synthetic construct
  misc_feature 1..21: note = Chemically synthesized nucleotide
  source 1..21: mol_type = other DNA
acgagcgggttcggcccattc

SEQ ID NO: 56 - DNA, 21 bp, synthetic construct
  misc_feature 1..21: note = Chemically synthesized nucleotide
  source 1..21: mol_type = other DNA
gggctacttgaggaccttgct

SEQ ID NO: 57 - DNA, 23 bp, synthetic construct
  misc_feature 1..23: note = Chemically synthesized nucleotide
  source 1..23: mol_type = other DNA
gacagcccttacagagtttggaa

SEQ ID NO: 58 - DNA, 20 bp, synthetic construct
  misc_feature 1..20: note = Chemically synthesized nucleotide
  source 1..20: mol_type = other DNA
cagggcctccatcccaggca

SEQ ID NO: 59 - DNA, 23 bp, synthetic construct
  misc_feature 1..23: note = Chemically synthesized nucleotide
  source 1..23: mol_type = other DNA
atctccctacttcctggctaatg

SEQ ID NO: 60 - DNA, 22 bp, synthetic construct
  misc_feature 1..22: note = Chemically synthesized nucleotide
  source 1..22: mol_type = other DNA
gcttggaacctgattggttgtc

SEQ ID NO: 61 - DNA, 27 bp, synthetic construct
  misc_feature 1..27: note = Chemically synthesized nucleotide
  source 1..27: mol_type = other DNA
agccttgatccttgggaatccaggaca

SEQ ID NO: 62 - DNA, 20 bp, synthetic construct
  misc_feature 1..20: note = Chemically synthesized nucleotide
  source 1..20: mol_type = other DNA
gcaaacaaaaaccactggcc

SEQ ID NO: 63 - DNA, 19 bp, synthetic construct
  misc_feature 1..19: note = Chemically synthesized nucleotide
  source 1..19: mol_type = other DNA
ggccacattccatgggttc

SEQ ID NO: 64 - DNA, 37 bp, synthetic construct
  misc_feature 1..37: note = Chemically synthesized nucleotide
  source 1..37: mol_type = other DNA
ctgttcctctaaaactggactccacagtaaatggaaa

SEQ ID NO: 65 - DNA, 26 bp, synthetic construct
  misc_feature 1..26: note = Chemically synthesized nucleotide
  source 1..26: mol_type = other DNA
caccatcgatgtcgacacgcctaggg

SEQ ID NO: 66 - DNA, 24 bp, synthetic construct
  misc_feature 1..24: note = Chemically synthesized nucleotide
  source 1..24: mol_type = other DNA
caccagtgtggccttgttagtctc

SEQ ID NO: 67 - DNA, 55 bp, synthetic construct
  misc_feature 1..55: note = Chemically synthesized nucleotide
  source 1..55: mol_type = other DNA
acactctttccctacacgacgctcttccgatctcagggtgactgatggcgaagac

SEQ ID NO: 68 - DNA, 57 bp, synthetic construct
  misc_feature 1..57: note = Chemically synthesized nucleotide
  source 1..57: mol_type = other DNA
gtgactggagttcagacgtgtgctcttccgatctcaccatcgatgtcgacacgccta

SEQ ID NO: 69 - DNA, 68 bp, synthetic construct
  misc_feature 1..68: note = Chemically synthesized nucleotide
  source 1..68: mol_type = other DNA
  misc_difference 30..35: note = n is a, c, g, t, unknown or other
aatgatacggcgaccaccgagatctacacnnnnnnacactctttccctacacgacgctcttccgatct

SEQ ID NO: 70 - DNA, 64 bp, synthetic construct
  misc_feature 1..64: note = Chemically synthesized nucleotide
  source 1..64: mol_type = other DNA
  misc_difference 25..30: note = n is a, c, g, t, unknown or other
caagcagaagacggcatacgagatnnnnnngtgactggagttcagacgtgtgctcttccgatct

SEQ ID NO: 71 - DNA, 30 bp, synthetic construct
  misc_feature 1..30: note = Chemically synthesized nucleotide
  source 1..30: mol_type = other DNA
cccatgtactctgcgttgataccactgctt

SEQ ID NO: 72 - DNA, 27 bp, synthetic construct
  misc_feature 1..27: note = Chemically synthesized nucleotide
  source 1..27: mol_type = other DNA
aagcagtggtatcaacgcagagtacat

SEQ ID NO: 73 - DNA, 24 bp, synthetic construct
  misc_feature 1..24: note = Chemically synthesized nucleotide
  source 1..24: mol_type = other DNA
caccagtgtggccttgttagtctc

SEQ ID NO: 74 - DNA, 57 bp, synthetic construct
  misc_feature 1..57: note = Chemically synthesized nucleotide
  source 1..57: mol_type = other DNA
gtgactggagttcagacgtgtgctcttccgatctaagcagtggtatcaacgcagagt

SEQ ID NO: 75 - DNA, 57 bp, synthetic construct
  misc_feature 1..57: note = Chemically synthesized nucleotide
  source 1..57: mol_type = other DNA
acactctttccctacacgacgctcttccgatctaaggtggaaacagggtgactgatg

SEQ ID NO: 76 - DNA, 67 bp, synthetic construct
  misc_feature 1..67: note = Chemically synthesized nucleotide
  source 1..67: mol_type = other DNA
  misc_difference 30..35: note = n is a, c, g, t, unknown or other
aatgatacggcgaccaccgagatctacacnnnnnnacactctttccctacacgacgctcttccgatc

SEQ ID NO: 77 - DNA, 64 bp, synthetic construct; identical to SEQ ID NO: 70
  misc_feature 1..64: note = Chemically synthesized nucleotide
  source 1..64: mol_type = other DNA
  misc_difference 25..30: note = n is a, c, g, t, unknown or other